European Patent Application EP 4 509 613 A1, published February 19, 2025. Title: METHOD FOR PRODUCING CULTURED MEAT. Applicant: Ajinomoto Co., Inc. Application WO PCT/JP2023/015195, filed April 14, 2023. The sequence listing filed with the application follows.

SEQUENCE LISTING (48 sequences)

SEQ ID NO: 1 - DNA, 1458 bp, Corynebacterium glutamicum
  source 1..1458: mol_type = genomic DNA
atggaaaacccttatgtcgctgcgctcgatgacgataaaaaagaagtcggcgcaataaaagaagcagaaaaagaacctgaaataggtcccatcagagctgccggacgagccataccgctgcgcacccgcatcattttgatcgtggtgggtatcgccgggcttggtttgctggtcaacgcgattgctgtttccagcctcatgcgtgaagtttcctatacccgcatggatcaagagctagagacctcgatggggacgtgggcgcataacgttgagctgtttaatttcgatggcgtccgccaagggccacccagcgattattatgtggccaaggtttttcctgatggatccagcattattttcaacgatgcacaatcggcacccaatctagctgaaaccaccatcggtactggtccacacactgtggatgctgctagcggttctgcctccaacactccgtggcgtgtgatggcggaaaagaacggtgacattatcaccgtggtgggtaaaagcatggggcgtgaaacaaacctgctgtaccgattggtgatggtgcagatgatcatcggcgcgctgattctggttgctattttgattacttcactcttcctagtcagacgctcgttgcggccgttgagagaagttgaagagaccgccaccaggattgcgggcggtgatttggatcgacgtgtcccgcagtggccaatgaccacagaagtcggacagctgtcgaatgccctcaatatcatgttggagcagctccaagcctcaattctgaccgcccagcaaaaagaagctcagatgcgccgattcgttggcgacgcctcccacgagctccgcacaccactgacctctgtgaagggcttcaccgagctgtattcatcaggtgcaacagatgatgccaactgggtcatgtccaagatcggtggcgaagcccaacgcatgagtgtgcttgtggaagacctcctgtcactgacgcgtgccgaaggccagcaaatggagaagcaccgcgttgacgtgctggaactcgcattggcagtacgcggatccatgcgagcagcctggccagatcgcaccgtcaacgtgtccaataaagccgagtccattccagttgttgaaggcgacccaacccgcctccaccaagttctcaccaacctggttgccaacggactcaaccacggcggaccggacgcggaagtcagcattgagatcaacaccgatgggcaaaacgtgaggattctcgtggcagacaacggtgtcggaatgtctgaagaagatgcccagcatatcttcgagcgtttctaccgcgccgattcctcccgctcacgcgcatccggcggatcgggcctcggccttgcgatcacgaaatccctggtcgaaggccacggcggcacagtcaccgtcgacagcgtgcaaggcgaaggcacggtgttcacgatcaccttgccggcggtttcttaa

SEQ ID NO: 2 - protein, 485 aa, Corynebacterium glutamicum
MENPYVAALDDDKKEVGAIKEAEKEPEIGPIRAAGRAIPLRTRIILIVVGIAGLGLLVNAIAVSSLMREVSYTRMDQELETSMGTWAHNVELFNFDGVRQGPPSDYYVAKVFPDGSSIIFNDAQSAPNLAETTIGTGPHTVDAASGSASNTPWRVMAEKNGDIITVVGKSMGRETNLLYRLVMVQMIIGALILVAILITSLFLVRRSLRPLREVEETATRIAGGDLDRRVPQWPMTTEVGQLSNALNIMLEQLQASILTAQQKEAQMRRFVGDASHELRTPLTSVKGFTELYSSGATDDANWVMSKIGGEAQRMSVLVEDLLSLTRAEGQQMEKHRVDVLELALAVRGSMRAAWPDRTVNVSNKAESIPVVEGDPTRLHQVLTNLVANGLNHGGPDAEVSIEINTDGQNVRILVADNGVGMSEEDAQHIFERFYRADSSRSRASGGSGLGLAITKSLVEGHGGTVTVDSVQGEGTVFTITLPAVS

SEQ ID NO: 3 - protein, 485 aa, Corynebacterium glutamicum
MENPYVAALDDENQEVGVKKEAEKEPEIGPIRAAGRAIPLRTRIILIVVGIAGLGLLVNAIAVSSLMREVSYTRMDQELETSMGTWAHNVELFNFDGVRQGPPSDYYVAKVFPDGSSIIFNDAQSAPDLAETTIGTGPHTVDAASGSASNTPWRVMAEKNGDIITVVGKSMGRETNLLYRLVMVQMIIGALILVAILITSLFLVRRSLRPLREVEETATRIAGGDLDRRVPQWPMTTEVGQLSNALNIMLEQLQASILTAQQKEAQMRRFVGDASHELRTPLTSVKGFTELYSSGATDDANWVMSKIGGEAQRMSVLVEDLLSLTRAEGQQMEKHRVDVLELALAVRGSMRAAWPDRTVNVSNKAESIPVVKGDPTRLHQVLTNLVANGLNHGGPDAEVSIEINTDGQNVRILVADNGVGMSEEDAQHIFERFYRADSSRSRASGGSGLGLAITKSLVEGHGGTVTVDSVQGEGTVFTITLPAVS

SEQ ID NO: 4 - protein, 485 aa, Corynebacterium glutamicum
MENPYVAALDDENQEVGVKKEAEKEPEIGPIRAAGRAIPLRTRIILIVVGIAGLGLLVNAIAVSSLMREVSYTRMDQELETSMGTWAHNVELFNFDGVRQGPPSDYYVAKVFPDGSSIIFNDAQSAPDLAETTIGTGPHTVDAASGSASNTPWRVMAEKNGDIITVVGKSMGRETNLLYRLVVVQMIIGALILVAILITSLFLVRRSLRPLREVEETATRIAGGDLDRRVPQWPMTTEVGQLSNALNIMLEQLQASILTAQQKEAQMRRFVGDASHELRTPLTSVKGFTELYSSGATDDANWVMSKIGGEAQRMSVLVEDLLSLTRAEGQQMEKHRVDVLELALAVRGSMRAAWPDRTVNVSNKAESIPVVEGDPTRLHQVLTNLVANGLNHGGPDAEVSIEINTDGQNVRILVADNGVGMSEEDAQHIFERFYRADSSRSRASGGSGLGLAITKSLVEGHGGTVTVDSVQGEGTVFTITLPAVS

SEQ ID NO: 5 - protein, 504 aa, Corynebacterium callunae
MENPYVAALDKNSNFGAKDTDSAVSDSTEVSQNNDGIGTPATAEPKVGPIRTAGRAMPLRTRIILLVVGIAGLGLLVNAVAVSSLMREVSYTRMDQDLESAMGTWVRNVELFNFDGVRQGPPSDYYVAKVFPDGSSIIFNDAESAPDLGQTTIGTGPHTVEAAEGSASSTHWRVMAAKNGDVITVVGKSMGRESTLLYRLVVVQMVIGVLILIAILIGSFFLVRRSLKPLREVEETASRIAGGELDRRVPQWPMTTEVGQLANALNIMLEQLQTSIMNAQQKEAQMRRFVGDASHELRTPLTSVKGFTELYSSGATQDADWVLSKIGGEAQRMSVLVEDLLSLTRAEGQQMEKHRVDMLELALAVRGSLKAAWPDRTVNVANRSENIPVVEGDPTRLHQVLTNLVANGLNHGGPEAEVNIQVETADDKVKILVIDNGVGMSKEDAEHIFERFYRADTSRSRASGGSGLGLAITKSLVEGHGGTITVDSELGKGTVFSIILPAAE

SEQ ID NO: 6 - protein, 458 aa, Corynebacterium crenatum
IGPIRAAGRAIPLRTRIILIVVGIAGLGLLVNAIAVSSLMREVSYTRMDQELETSMGTWAHNVELFNFDGVRQGPPSDYYVAKVFPDGSSIIFNDAQSAPDLAETTIGTGPHTVDAASGSASNTPWRVMAEKNGDIITVVGKSMGRETNLLYRLVMVQMIIGALILVAILITSLFLVRRSLRPLREVEETATRIAGGDLDRRVPQWPMTTEVGQLSNALNIMLEQLQASILSAQQKEAQMRRFVGDASHELRTPLTSVKGFTELYSSGATDDANWVMSKIGGEAQRMSVLVEDLLSLTRAEGQQMEKHRVDVLELALAVRGSMRAAWPDRTVNVSNKAASIPVVEGDPTRLHQVLTNLVANGLNHGGPDAEVSIEINTDGQNVRILVADNGVGMSEEDAQHIFERFYRADSSRSRASGGSGLGLAITKSLVEGHGGTVTVDSVQGEGTVFTITLPAVS

SEQ ID NO: 7 - protein, 471 aa, Corynebacterium efficiens
MTAPENPHAQVTPVGRFRQAARGVPLRTRIILLVVGIAGLGLLVNAIAVSSLMREVSYSRMDQELESAMNSWAQTAELFGSITLGPPSDYYVVRIFPDGSHMVFNQSDSAPDLGETTIGIGPHTASAAPGSSSSVPWRVIAISDNGTITVVGKSLAPESMLLYRLVIVQLVIGMLIVVAILLSSLYLVNRSLRPLREVEKTAKSIAGGDLDRRVPQWPMTTEVGQLANALNIMLEQLQASILSAQEKESQMRRFVGDASHELRTPLTSVKGYSELYHSGATRDADWVLSKISGEAQRMSVLVEDLLSLTRAEGQQMEKRPVDVLELSLSVASSMRAAWPERSITVVNKTGSLPVVEGDATRLHQVLTNLVNNGLNHGGPDASVEIEISAEGGSVLVRVVDDGVGMTAEDAQHIFERFYRTDTSRSRASGGSGLGLAITKSLVEGHRGTITVDSEVGEGTVFTITLPSRMED

SEQ ID NO: 8 - DNA, 708 bp, Corynebacterium glutamicum
  source 1..708: mol_type = genomic DNA
atggacaaccagtctgacggacaaatccgcgtactcgtcgttgatgacgagccaaacatcgtcgagctgctcaccgtaagccttaaattccaaggcttcgcagtgatgaccgccaacgatggcaatgaagccctgaagattgctcgtgagttccgtccagacgcatacatcctcgatgtcatgatgccaggaatggacggcttcgagctgctgaccaagctgcgcggcgaaggccttgacagcccagttctgtacctcaccgcaaaggatgccgtggagcaccgcatccacggcctgaccatcggcgctgacgactacgtgaccaagcctttctccctggaagaagtaatcacccgcctgcgcgtgattcttcgtcgcggtggagcagttgaagaagacacctcaacttccctgcagtacgcagacctcaccctcaacgatgaaacccacgaggtcaccaaggctggcgaactgatcgatctttccccaactgaattcaacctcctgcgctacctcatgctcaacgctgaagtggtgctgtccaaggcaaagatcctggataacgtgtggcactacgattttggtggcgacggcaacgtcgtggaatcctacatctcctacctgcgccgcaaggtggacacccaggatccgcagctaattcagactgttcgtggcgttggatatgttctgcgcaccccacgtagctaa

SEQ ID NO: 9 - protein, 235 aa, Corynebacterium glutamicum
MDNQSDGQIRVLVVDDEPNIVELLTVSLKFQGFAVMTANDGNEALKIAREFRPDAYILDVMMPGMDGFELLTKLRGEGLDSPVLYLTAKDAVEHRIHGLTIGADDYVTKPFSLEEVITRLRVILRRGGAVEEDTSTSLQYADLTLNDETHEVTKAGELIDLSPTEFNLLRYLMLNAEVVLSKAKILDNVWHYDFGGDGNVVESYISYLRRKVDTQDPQLIQTVRGVGYVLRTPRS

SEQ ID NO: 10 - DNA, 1500 bp, Corynebacterium glutamicum
  source 1..1500: mol_type = genomic DNA
atgtttaacaaccgtatccgcactgcagctctcgctggtgcaatcgcaatctccaccgcagcttccggcgtagctatcccagcattcgctcaggagaccaacccaaccttcaacatcaacaacggcttcaacgatgctgatggatccaccatccagccagttgagccagttaaccacaccgaggaaaccctccgcgacctgactgactccaccggcgcttacctggaagagttccagtacggcaacgttgaggaaatcgttgaagcatacctgcaggttcaggcttccgcagacggattcgatccttctgagcaggctgcttacgaggctttcgaggctgctcgcgttcgtgcatcccaggagctcgcggcttccgctgagaccatcactaagacccgcgagtccgttgcttacgcactcaaggctgaccgcgaagctaccgcagctttcgaggcttacctcagcgctcttcgtcaggtttcagtcatcaacgatctgatcgctgatgctaacgccaagaacaagactgactttgcagagatcgagctctacgatgttctttacaccgacgccgacatctctggcgatgctccacttcttgctcctgcatacaaggagctgaaggaccttcaggctgaggttgacgcagacttcgagtggttgggcgagttcgcaattgataacaatgaagacaactacgtcattcgtactcacatccctgctgtagaggcactcaaggcagcgatcgattcactggtcgacaccgttgagccacttcgtgcagacgctatcgctaagaacatcgaggctcagaagtctgacgttctggttccccagctcttcctcgagcgtgcaactgcacagcgcgacaccctgcgtgttgtagaggcaatcttctctacctctgctcgttacgttgaactctacgagaacgtcgagaacgttaacgttgagaacaagacccttcgccagcactactcttccctgatccctaacctcttcatcgcagcggttggcaacatcaacgagctcaacaatgcagatcaggctgcacgtgagctcttcctcgattgggacaccgacctcaccaccaacgatgaggacgaagcttactaccaggctaagctcgacttcgctatcgagacctacgcaaagatcctgatcaacggtgaagtttggcaggagccactcgcttacgtccagaacctggatgcaggcgcacgtcaggaagcagctgaccgcgaagcagagcgcgcagctgacgcagcataccgcgctgagcagctccgcatcgctcaggaagcagctgacgctcagaaggctctcgctgaggctcttgctaatgcaggcaacaacgacaacggtggcgacaactcctccgacgacaagggaaccggttcttccgacatcggaacctggggacctttcgcagcaattgcagctatcatcgcagcaatcgcagctatcttcccattcctctccggtatcgttaagttctaa

SEQ ID NO: 11 - protein, 499 aa, Corynebacterium glutamicum
MFNNRIRTAALAGAIAISTAASGVAIPAFAQETNPTFNINNGFNDADGSTIQPVEPVNHTEETLRDLTDSTGAYLEEFQYGNVEEIVEAYLQVQASADGFDPSEQAAYEAFEAARVRASQELAASAETITKTRESVAYALKADREATAAFEAYLSALRQVSVINDLIADANAKNKTDFAEIELYDVLYTDADISGDAPLLAPAYKELKDLQAEVDADFEWLGEFAIDNNEDNYVIRTHIPAVEALKAAIDSLVDTVEPLRADAIAKNIEAQKSDVLVPQLFLERATAQRDTLRVVEAIFSTSARYVELYENVENVNVENKTLRQHYSSLIPNLFIAAVGNINELNNADQAARELFLDWDTDLTTNDEDEAYYQAKLDFAIETYAKILINGEVWQEPLAYVQNLDAGARQEAADREAERAADAAYRAEQLRIAQEAADAQKALAEALANAGNNDNGGDNSSDDKGTGSSDIGTWGPFAAIAAIIAAIAAIFPFLSGIVKF

SEQ ID NO: 12 - DNA, 318 bp, Corynebacterium glutamicum
  source 1..318: mol_type = genomic DNA
atgtccctcggaccatgggaaattggaatcattgtcctgctgatcatcgtgctgttcggcgcgaagaagctgcctgatgcagctcgttccatcggccgttccatgcgcatcttcaagtctgaagtcaaagaaatgaacaaggacggcgataccccagaacaacagcagcagcctcagcagcagattgcgcccaaccagatcgaggctcctcagccaaactttgagcagcactaccagggacagcaggttcagcagcctcagaaccctcagacccctgactaccgtcagaactacgaggatccaaaccgcacctcttaa

SEQ ID NO: 13 - protein, 105 aa, Corynebacterium glutamicum
MSLGPWEIGIIVLLIIVLFGAKKLPDAARSIGRSMRIFKSEVKEMNKDGDTPEQQQQPQQQIAPNQIEAPQPNFEQHYQGQQVQQPQNPQTPDYRQNYEDPNRTS

SEQ ID NO: 14 - DNA, 471 bp, Corynebacterium glutamicum
  source 1..471: mol_type = genomic DNA
atgttttctagcgtgggttggggagagatcttcctcttagtcgttgtgggccttgttgtcatcggcccggaacggttgcctcgtttgatccaggacgcacgcgctgcgctgctcgctgcacgtaccgctatcgacaatgcaaagcagtcgttggacagtgattttggttcggaatttgatgaaatccgaaagccactaacccaggttgcacagtacagccggatgagccccaagacggccatcactaaggcgttatttgataatgattcctcgttcctggatgactttgatccaaagaagatcatggccgaaggaacagaaggcgaagctcagcgcaacaagcaggcagctgacaacaatgcgaatgtggtggaacgtccagctgatggttccaccgcacgcccaacgcaaaacgatccaaaagacggcccgaattactcaggtggcgtctcttggaccgatattatttag

SEQ ID NO: 15 - protein, 156 aa, Corynebacterium glutamicum
MFSSVGWGEIFLLVVVGLVVIGPERLPRLIQDARAALLAARTAIDNAKQSLDSDFGSEFDEIRKPLTQVAQYSRMSPKTAITKALFDNDSSFLDDFDPKKIMAEGTEGEAQRNKQAADNNANVVERPADGSTARPTQNDPKDGPNYSGGVSWTDII

SEQ ID NO: 16 - DNA, 945 bp, Corynebacterium glutamicum
  source 1..945: mol_type = genomic DNA
atgtccattgttgagcacatcaaagagtttcgacgccgacttcttatcgctctggcgggcatcctcgtgggcaccattatcggctttatttggtacgatttctcattttggcagatccccactttgggcgagctgctgagggatccgtactgttctctgcctgctgaatcccgctgggccatgagcgactcagaggaatgtcgactgctcgcaaccggcccgtttgatccattcatgcttcgccttaaagtagcggcgttggtgggtatggttcttggctcacccgtgtggctgagccagctgtggggctttatcaccccaggtttgatgaagaatgagcgccgttacaccgcaatcttcgtcacgattgctgttgtgctgtttgtcggcggtgctgttcttgcgtacttcgtcgttgcatatggtttggagttcctccttaccattggtggagacacccaggcagcggccctgactggtgataagtacttcggattcttgctcgcgttgttggcgattttcggcgtgagcttcgaagttccactggtgatcggcatgctcaacattgtgggtatcttgccttacgatgccattaaagataagcgacgcatgatcatcatgattttgttcgtgttcgctgctttcatgacacccggccaggatcctttcaccatgttggtgttggcgctttcactcaccgttctggtagagcttgccctgcagttctgtcgtttcaacgacaaacgccgggacaagaagcgcccagaatggcttgatggcgatgacctctctgcatcaccactggatacttctgctggtggagaagatgctccaagcccagtcgaaaccccagaggcggtggagccttcgcggatgctgaacccaagtggggaggcgtcgataagctataaacccgggcgcgccgacttcggtgacgtgctctag

SEQ ID NO: 17 - protein, 314 aa, Corynebacterium glutamicum
MSIVEHIKEFRRRLLIALAGILVGTIIGFIWYDFSFWQIPTLGELLRDPYCSLPAESRWAMSDSEECRLLATGPFDPFMLRLKVAALVGMVLGSPVWLSQLWGFITPGLMKNERRYTAIFVTIAVVLFVGGAVLAYFVVAYGLEFLLTIGGDTQAAALTGDKYFGFLLALLAIFGVSFEVPLVIGMLNIVGILPYDAIKDKRRMIIMILFVFAAFMTPGQDPFTMLVLALSLTVLVELALQFCRFNDKRRDKKRPEWLDGDDLSASPLDTSAGGEDAPSPVETPEAVEPSRMLNPSGEASISYKPGRADFGDVL

SEQ ID NO: 18 - protein, 39 aa, Escherichia coli
MNNNDLFQASRRRFLAQLGGLTVAGMLGPSLLTPRRATA

SEQ ID NO: 19 - protein, 27 aa, Escherichia coli
MSLSRRQFIQASGIALCAGAVPLKASA

SEQ ID NO: 20 - protein, 48 aa, Bacillus subtilis
MAYDSRFDEWVQKLKEESFQNNTFDRRKFIQGAGKIAGLSLGLTIAQS

SEQ ID NO: 21 - protein, 34 aa, Bacillus subtilis
MKFVKRRTTALVTTLMLSVTSLFALQPSAKAAEH

SEQ ID NO: 22 - protein, 30 aa, Arthrobacter globiformis
MMNLSRRTLLTTGSAATLAYALGMAGSAQA

SEQ ID NO: 23 - protein, 7 aa, synthetic construct
  REGION 1..7: note = Twin-Arginine Motif
  SITE 1: note = misc_feature - Xaa can be any naturally occurring amino acid
  SITE 4: note = misc_feature - Xaa can be any naturally occurring amino acid
XRRXFLK

SEQ ID NO: 24 - skipped

SEQ ID NO: 25 - protein, 43 aa, Corynebacterium glutamicum
MRDTAFRSIKAKAQAKRRSLWIAAGAVPTAIALTMSLAPMASA

SEQ ID NO: 26 - protein, 30 aa, Corynebacterium glutamicum
MFNNRIRTAALAGAIAISTAASGVAIPAFA

SEQ ID NO: 27 - protein, 25 aa, Corynebacterium stationis
MKRMKSLAAALTVAGAMLAAPVATA

SEQ ID NO: 28 - protein, 469 aa, Corynebacterium glutamicum
QETNPTFNINNGFNDADGSTIQPVEPVNHTEETLRDLTDSTGAYLEEFQYGNVEEIVEAYLQVQASADGFDPSEQAAYEAFEAARVRASQELAASAETITKTRESVAYALKADREATAAFEAYLSALRQVSVINDLIADANAKNKTDFAEIELYDVLYTDADISGDAPLLAPAYKELKDLQAEVDADFEWLGEFAIDNNEDNYVIRTHIPAVEALKAAIDSLVDTVEPLRADAIAKNIEAQKSDVLVPQLFLERATAQRDTLRVVEAIFSTSARYVELYENVENVNVENKTLRQHYSSLIPNLFIAAVGNINELNNADQAARELFLDWDTDLTTNDEDEAYYQAKLDFAIETYAKILINGEVWQEPLAYVQNLDAGARQEAADREAERAADAAYRAEQLRIAQEAADAQKALAEALANAGNNDNGGDNSSDDKGTGSSDIGTWGPFAAIAAIIAAIAAIFPFLSGIVKF

SEQ ID NO: 29-31 - skipped (3 entries)

SEQ ID NO: 32 - protein, 6 aa, Corynebacterium glutamicum
QETNPT

SEQ ID NO: 33 - protein, 6 aa, Corynebacterium glutamicum
QETGTY

SEQ ID NO: 34 - protein, 6 aa, Corynebacterium glutamicum
QETTVT

SEQ ID NO: 35 - protein, 6 aa, Corynebacterium glutamicum
QETPVT

SEQ ID NO: 36 - protein, 6 aa, Corynebacterium glutamicum
QETAVT

SEQ ID NO: 37 - protein, 4 aa, synthetic construct
  REGION 1..4: note = Factor Xa
IEGR

SEQ ID NO: 38 - protein, 6 aa, synthetic construct
  REGION 1..6: note = ProTEV
ENLYFQ

SEQ ID NO: 39 - DNA, 1563 bp, Corynebacterium glutamicum
  source 1..1563: mol_type = genomic DNA
gtgagccaagccctacctgttcgtgaccaggggcgggaccaggggattttcgctggtactctcccgcccgcaccgccaaagttcaagtggacccgcctggatacctatacctgggcgatcatcgcggtgtttgctttagtcacgcgttttacaggtttgagcagtgcaaccgcctcaggcaccccagtttttgatgaaaaacactacgtcccacaagcctgggacatggtccgctcctggatcaaccccatcaccggcggcattgaatccaaccccggatacggactcgtcgttcacccaccgttggccaaacaacttgaagcactcggtgaatgggtcttcggatacacccccctcggctggcgcatcatggtcgccattttcggaacactcaccattttcgccatcatggcaatcgcacggcgcctcagcggatccaccattgtgactttcatcgccggaattctcgcgcttgccgacggcgtcctcctcgtctcatcacgcttcggcatgctggacatcttccttgttttcttcatcaccgcagcagcatgggcattgatccgagatcaccaacaaatgcaccaacgcctcaacgatttactcctcaccaacggccaaatcaccaaagactttggcccccgattcggcttccgatggtggcgtttcaccacaggtgtattccttggtctcgcgctctccgtcaaatggtccggactgtactacatcgcattcttcggcctgaccagcgtgttcctagacttgtggctgcgcaaacgctacggcgtccgacgctacgtcaccggcaccctaaaaaatgacgtcatcccagcgctcggctccttggtgatcatccctgccctgctttatatctggagctggcgagcctggttcgcctccgaaacctccgtctaccgccacgccaaaacagacggcaccatcacagaagactccatcctgcagctcttccctgaatcaattgcgggctggatccactatcacatcagcgtcctggaattccacggctcactgaccacatcctcaggtcacagccacccctgggattccaagccgtgggcctggcttgtctccggtcgacccatcctctacttctcctccaccgacatctcctgcgacgttggcggcacctgccgacgcatgatctacctcttcggcacgcccgccatttggtggctgacagtcccagtcattctgtgggcgctgtggtctttcttcgcacgtcggagtcgtggctatattgtcccactagtggccttcgctgcaggatttttgccgtggcttgcagcatacgaccgccaaatgtacttcttctacgccaccgcattggtgccattcaccatcatcatgttggcactcgcctgcggtgaactgtggggccgtggaaaaatgacccccactggcttaacccgcggatcaatggcagtggtcacctacatttccctcgtggtgatgatgtttctcgcgttttcgccactgttttacggatttgtcatcccagattatgtctacgaatccttgatgtggttcccaagctggcgctaa

SEQ ID NO: 40 - protein, 520 aa, Corynebacterium glutamicum
MSQALPVRDQGRDQGIFAGTLPPAPPKFKWTRLDTYTWAIIAVFALVTRFTGLSSATASGTPVFDEKHYVPQAWDMVRSWINPITGGIESNPGYGLVVHPPLAKQLEALGEWVFGYTPLGWRIMVAIFGTLTIFAIMAIARRLSGSTIVTFIAGILALADGVLLVSSRFGMLDIFLVFFITAAAWALIRDHQQMHQRLNDLLLTNGQITKDFGPRFGFRWWRFTTGVFLGLALSVKWSGLYYIAFFGLTSVFLDLWLRKRYGVRRYVTGTLKNDVIPALGSLVIIPALLYIWSWRAWFASETSVYRHAKTDGTITEDSILQLFPESIAGWIHYHISVLEFHGSLTTSSGHSHPWDSKPWAWLVSGRPILYFSSTDISCDVGGTCRRMIYLFGTPAIWWLTVPVILWALWSFFARRSRGYIVPLVAFAAGFLPWLAAYDRQMYFFYATALVPFTIIMLALACGELWGRGKMTPTGLTRGSMAVVTYISLVVMMFLAFSPLFYGFVIPDYVYESLMWFPSWR

SEQ ID NO: 41 - DNA, 26 bp, synthetic construct
  source 1..26: mol_type = other DNA
  misc_feature 3..26: note = primer
gtttcgtacctaaaccgacccgaacc

SEQ ID NO: 42 - DNA, 24 bp, synthetic construct
  source 1..24: mol_type = other DNA
  misc_feature 4..24: note = primer
tcggttgattgtagagccttggcg

SEQ ID NO: 43 - DNA, 46 bp, synthetic construct
  source 1..46: mol_type = other DNA
  misc_feature 5..46: note = primer
gccaaggctctacaatcaaccgatggccgaaccaagtgaccaatgc

SEQ ID NO: 44 - DNA, 25 bp, synthetic construct
  source 1..25: mol_type = other DNA
  misc_feature 6..25: note = primer
aagctccggcattgattccgttacc

SEQ ID NO: 45 - DNA, 468 bp, Bos taurus
  source 1..468: mol_type = genomic DNA
atggcagcaggctccatcacgaccttgccagctcttccagaagatggcggatctggagcctttccaccaggacacttcaaggaccccaaacgcctctactgcaagaatggcgggttctttctgcgcattcatcctgatggccgagttgacggtgttcgcgaaaagagcgacccgcacatcaaactgcagcttcaagctgaggaacgtggtgtggtgagcatcaaaggtgtctgtgccaaccggtatctggcgatgaaggaggatggccgtttgctggcatccaagtgcgtaaccgatgagtgcttcttcttcgaacgtctggagtccaacaactacaacacctatcgctcacgcaagtactcctcttggtacgtcgctctgaaacgcacaggccagtacaagcttggtcccaaaactgggcctggtcagaaggcgattctcttcctcccgatgtccgccaagtcgtaa

SEQ ID NO: 46 - protein, 155 aa, Bos taurus
MAAGSITTLPALPEDGGSGAFPPGHFKDPKRLYCKNGGFFLRIHPDGRVDGVREKSDPHIKLQLQAEERGVVSIKGVCANRYLAMKEDGRLLASKCVTDECFFFERLESNNYNTYRSRKYSSWYVALKRTGQYKLGPKTGPGQKAILFLPMSAKS

SEQ ID NO: 47 - DNA, 585 bp, Bos taurus
  source 1..585: mol_type = genomic DNA
atgaacaataacgatctctttcaggcatcacgtcggcgttttctggcacaactcggcggcttaaccgtcgccgggatgctggggccgtcattgttaacgccgcgacgtgcgactgcgatggcagcaggctccatcacgaccttgccagctcttccagaagatggcggatctggagcctttccaccaggacacttcaaggaccccaaacgcctctactgcaagaatggcgggttctttctgcgcattcatcctgatggccgagttgacggtgttcgcgaaaagagcgacccgcacatcaaactgcagcttcaagctgaggaacgtggtgtggtgagcatcaaaggtgtctgtgccaaccggtatctggcgatgaaggaggatggccgtttgctggcatccaagtgcgtaaccgatgagtgcttcttcttcgaacgtctggagtccaacaactacaacacctatcgctcacgcaagtactcctcttggtacgtcgctctgaaacgcacaggccagtacaagcttggtcccaaaactgggcctggtcagaaggcgattctcttcctcccgatgtccgccaagtcgtaa

SEQ ID NO: 48 - protein, 194 aa, Bos taurus
MNNNDLFQASRRRFLAQLGGLTVAGMLGPSLLTPRRATAMAAGSITTLPALPEDGGSGAFPPGHFKDPKRLYCKNGGFFLRIHPDGRVDGVREKSDPHIKLQLQAEERGVVSIKGVCANRYLAMKEDGRLLASKCVTDECFFFERLESNNYNTYRSRKYSSWYVALKRTGQYKLGPKTGPGQKAILFLPMSAKS